European Patent Specification EP 3 853 256 B1, published August 21, 2024. Title: Dual acting CD1d immunoglobulin. Applicant: LAVA Therapeutics. The sequence listing filed with the application follows.

SEQUENCE LISTING (88 sequences)

SEQ ID NO: 1 - protein, 5 aa, Artificial Sequence
  antibody sequence
DNVMG

SEQ ID NO: 2 - protein, 16 aa, Artificial Sequence
  antibody sequence
TIRTGGSTNYADSVKG

SEQ ID NO: 3 - protein, 11 aa, Artificial Sequence
  antibody sequence
TIPVPSTPYDY

SEQ ID NO: 4 - protein, 119 aa, Artificial Sequence
  antibody sequence
QVQLVESGGGLVQAGGSLRLSCAASGSMFSDNVMGWYRQAPGKQRELVATIRTGGSTNYADSVKGRFTISRDNAKNTVYLQMNSLKPEDTAVYYCRHTIPVPSTPYDYWGQGTQVTVSS

SEQ ID NO: 5 - protein, 5 aa, Artificial Sequence
  antibody sequence
SYAMG

SEQ ID NO: 6 - protein, 17 aa, Artificial Sequence
  antibody sequence
AISWSGGTTYYADSVKG

SEQ ID NO: 7 - protein, 16 aa, Artificial Sequence
  antibody sequence
SLDCSGPGCHTAEYDY

SEQ ID NO: 8 - protein, 5 aa, Artificial Sequence
  antibody sequence
EYAMG

SEQ ID NO: 9 - protein, 17 aa, Artificial Sequence
  antibody sequence
AISWTGSKTYYADSVKG

SEQ ID NO: 10 - protein, 16 aa, Artificial Sequence
  antibody sequence
SSDCSGPGCHTEEYDY

SEQ ID NO: 11 - protein, 5 aa, Artificial Sequence
  antibody sequence
SYAMG

SEQ ID NO: 12 - protein, 17 aa, Artificial Sequence
  antibody sequence
AVSWSGGSTYYADSVKG

SEQ ID NO: 13 - protein, 16 aa, Artificial Sequence
  antibody sequence
SQDCSGPGCYTNEYDS

SEQ ID NO: 14 - protein, 5 aa, Artificial Sequence
  antibody sequence
NYAMA

SEQ ID NO: 15 - protein, 17 aa, Artificial Sequence
  antibody sequence
AVSWSGGRTYYADSVKG

SEQ ID NO: 16 - protein, 16 aa, Artificial Sequence
  antibody sequence
SLSCSGPGCSLEEYDY

SEQ ID NO: 17 - protein, 5 aa, Artificial Sequence
  antibody sequence
NYAMG

SEQ ID NO: 18 - protein, 17 aa, Artificial Sequence
  antibody sequence
VISWSGGSTYYADSVKG

SEQ ID NO: 19 - protein, 18 aa, Artificial Sequence
  antibody sequence
QFSGASTVVAGTALDYDY

SEQ ID NO: 20 - protein, 5 aa, Artificial Sequence
  antibody sequence
NYGMG

SEQ ID NO: 21 - protein, 17 aa, Artificial Sequence
  antibody sequence
GISWSGGSTDYADSVKG

SEQ ID NO: 22 - protein, 17 aa, Artificial Sequence
  antibody sequence
VFSGAETAYYPSDDYDY

SEQ ID NO: 23 - protein, 5 aa, Artificial Sequence
  antibody sequence
NYGMG

SEQ ID NO: 24 - protein, 17 aa, Artificial Sequence
  antibody sequence
GISWSGGSTDYADSVKG

SEQ ID NO: 25 - protein, 17 aa, Artificial Sequence
  antibody sequence
VFSGAETAYYPSDDYDY

SEQ ID NO: 26 - protein, 5 aa, Artificial Sequence
  antibody sequence
NYGMG

SEQ ID NO: 27 - protein, 17 aa, Artificial Sequence
  antibody sequence
GISWSGGSTDYADSVKG

SEQ ID NO: 28 - protein, 17 aa, Artificial Sequence
  antibody sequence
VFSGAETAYYPSDDYDY

SEQ ID NO: 29 - protein, 5 aa, Artificial Sequence
  antibody sequence
NYGMG

SEQ ID NO: 30 - protein, 17 aa, Artificial Sequence
  antibody sequence
GITWSGGSTHYADLVKG

SEQ ID NO: 31 - protein, 17 aa, Artificial Sequence
  antibody sequence
VFSGAETAYYPSTEYDY

SEQ ID NO: 32 - protein, 5 aa, Artificial Sequence
  antibody sequence
NYGMG

SEQ ID NO: 33 - protein, 17 aa, Artificial Sequence
  antibody sequence
GISWSGGSTYYADSVKG

SEQ ID NO: 34 - protein, 17 aa, Artificial Sequence
  antibody sequence
VFSGAETAQYPSYDYDY

SEQ ID NO: 35 - protein, 5 aa, Artificial Sequence
  antibody sequence
NYAMG

SEQ ID NO: 36 - protein, 17 aa, Artificial Sequence
  antibody sequence
AISWSGGSTSYADSVKG

SEQ ID NO: 37 - protein, 21 aa, Artificial Sequence
  antibody sequence
QFSGADYGFGRLGIRGYEYDY

SEQ ID NO: 38 - protein, 5 aa, Artificial Sequence
  antibody sequence
NYAMG

SEQ ID NO: 39 - protein, 17 aa, Artificial Sequence
  antibody sequence
AISWSGGSTYYADSVKG

SEQ ID NO: 40 - protein, 21 aa, Artificial Sequence
  antibody sequence
MFSGSESQLVVVITNLYEYDY

SEQ ID NO: 41 - protein, 5 aa, Artificial Sequence
  antibody sequence
NYAMG

SEQ ID NO: 42 - protein, 17 aa, Artificial Sequence
  antibody sequence
TISWSGGSTYYADSVKG

SEQ ID NO: 43 - protein, 18 aa, Artificial Sequence
  antibody sequence
AFSGSDYANTKKEVEYDY

SEQ ID NO: 44 - protein, 5 aa, Artificial Sequence
  antibody sequence
DYCIA

SEQ ID NO: 45 - protein, 17 aa, Artificial Sequence
  antibody sequence
CITTSDGSTYYADSVKG

SEQ ID NO: 46 - protein, 18 aa, Artificial Sequence
  antibody sequence
YFGYGCYGGAQDYRAMDY

SEQ ID NO: 47 - protein, 5 aa, Artificial Sequence
  antibody sequence
RYTMG

SEQ ID NO: 48 - protein, 17 aa, Artificial Sequence
  antibody sequence
AISWSGGRTNFAGSVKG

SEQ ID NO: 49 - protein, 13 aa, Artificial Sequence
  antibody sequence
DWLPVPGRESYDY

SEQ ID NO: 50 - protein, 5 aa, Artificial Sequence
  antibody sequence
NYAMG

SEQ ID NO: 51 - protein, 17 aa, Artificial Sequence
  antibody sequence
AISWSGGMTDHADSVKG

SEQ ID NO: 52 - protein, 21 aa, Artificial Sequence
  antibody sequence
AFAGDIPYGSSWYGDPTTYDY

SEQ ID NO: 53 - protein, 5 aa, Artificial Sequence
  antibody sequence
TFSMA

SEQ ID NO: 54 - protein, 17 aa, Artificial Sequence
  antibody sequence
AINWSGGSTRYADSVSD

SEQ ID NO: 55 - protein, 15 aa, Artificial Sequence
  antibody sequence
RRGGIYYSTQNDYDY

SEQ ID NO: 56 - protein, 5 aa, Artificial Sequence
  antibody sequence
DYRMG

SEQ ID NO: 57 - protein, 17 aa, Artificial Sequence
  antibody sequence
TISWSGGLTYYADSVKG

SEQ ID NO: 58 - protein, 14 aa, Artificial Sequence
  antibody sequence
GGGYAGGTYYHPEE

SEQ ID NO: 59 - protein, 125 aa, Artificial Sequence
  antibody sequence
EVQLVESGGGLVQAGGSLRLSCTASGRTFSSYAMGWFRQAPGKEREFVAAISWSGGTTYYADSVKGRFTISRDNAKNTVSLQMNSLKPEDTAVYFCAASLDCSGPGCHTAEYDYWGQGTQVTVSS

SEQ ID NO: 60 - protein, 125 aa, Artificial Sequence
  antibody sequence
EVQLVESGGGLVQAGGSLRLSCAATGRTFSEYAMGWFRQAPGKEREFAAAISWTGSKTYYADSVKGRFTISRDNAKNTVYLQMNSLKPEDTAVYYCAASSDCSGPGCHTEEYDYWGQGTQVTVSS

SEQ ID NO: 61 - protein, 125 aa, Artificial Sequence
  antibody sequence
EVQLVESGGGLVQAGGSLRLSCAASGRTFSSYAMGWFRQAPGKEREFVAAVSWSGGSTYYADSVKGRFTISRDNARNTVYLQMNSLNPEDTAVYYCAASQDCSGPGCYTNEYDSWGQGTQVTVSS

SEQ ID NO: 62 - protein, 125 aa, Artificial Sequence
  antibody sequence
EVQLVESGGGLVQPGGSLRLSCAASGSIFSNYAMAWFRQAPEKERDFLAAVSWSGGRTYYADSVKGRFTISRDNAKNTVNLQMNSLKPEDTAVYYCAASLSCSGPGCSLEEYDYWGQGTQVTVSS

SEQ ID NO: 63 - protein, 127 aa, Artificial Sequence
  antibody sequence
EVQLVESGGGLVQAGGSLRLSCAASGRPFSNYAMGWFRQAPGKEREFVTVISWSGGSTYYADSVKGRFTISRDNAKNTVYLQMNSLKPEDTAVYYCAAQFSGASTVVAGTALDYDYWGQGTRVTVSS

SEQ ID NO: 64 - protein, 126 aa, Artificial Sequence
  antibody sequence
EVQLVESGGGLVQAGGSLRLSCAASGRPFSNYGMGWFRQAPGKKREFVAGISWSGGSTDYADSVKGRLTISRDNAKNTVYLQMNSLKPEDTAVYYCAAVFSGAETAYYPSDDYDYWGQGTQVTVSS

SEQ ID NO: 65 - protein, 126 aa, Artificial Sequence
  antibody sequence
EVQLVESGGGLVQAGGSLRLSCAASGRPFSNYGMGWFRQAPGKKREFVAGISWSGGSTDYADSVKGRFTISRDNAKNTVYLQMNSLKPEDTAVYYCAAVFSGAETAYYPSDDYDYWGQGTQVTVSS

SEQ ID NO: 66 - protein, 126 aa, Artificial Sequence
  antibody sequence
EVQLVESGGGLVQAGGSLRLSCAASGRPFSNYGMGWFRQAPGKKRESVAGISWSGGSTDYADSVKGRFTISRDNAKNTVYLQMNSLKPEDTAVYYCAAVFSGAETAYYPSDDYDYWGQGTQVTVSS

SEQ ID NO: 67 - protein, 126 aa, Artificial Sequence
  antibody sequence
EVQLVESGGGLVQAGGSLRLSCAVSGRPFSNYGMGWFRQAPGKEREFVAGITWSGGSTHYADLVKGRFTISRDNAKNTVHLQMNSLKPEDTAVYYCAAVFSGAETAYYPSTEYDYWGQGTQVTVSS

SEQ ID NO: 68 - protein, 126 aa, Artificial Sequence
  antibody sequence
EVQLVESGGGLVQAGGSLRLSCAASGRPFNNYGMGWFRQAPGKEREFVAGISWSGGSTYYADSVKGRFTISRDNAKNTVYLQMNSLKPEDTAVYYCAAVFSGAETAQYPSYDYDYWGQGTQVTVSS

SEQ ID NO: 69 - protein, 130 aa, Artificial Sequence
  antibody sequence
EVQLVESGGGLVQAGGSLRLSCAASGRPFSNYAMGWFRQAPGKEREFVAAISWSGGSTSYADSVKGRFTISRDNAKNTVYLQMNSPKPEDTAIYYCAAQFSGADYGFGRLGIRGYEYDYWGQGTQVTVSS

SEQ ID NO: 70 - protein, 130 aa, Artificial Sequence
  antibody sequence
EVQLVESGGGLVQAGGSLRLSCAASGRTFSNYAMGWFRQAPGKEREFVAAISWSGGSTYYADSVKGRFTISRDNAKNTVYLQMNSLKPEDTAVYYCAAMFSGSESQLVVVITNLYEYDYWGQGTQVTVSS

SEQ ID NO: 71 - protein, 127 aa, Artificial Sequence
  antibody sequence
EVQLVESGGGLVQAGGSLRLSCAASGRTFSNYAMGWFRQAPGKEREFVATISWSGGSTYYADSVKGRFTISRDNAKNTVYLQMNSLKPEDTAVYYCAAAFSGSDYANTKKEVEYDYWGQGTQVTVSS

SEQ ID NO: 72 - protein, 127 aa, Artificial Sequence
  antibody sequence
EVQLVESGGGLVQAGGSLRLSCAASGFTFDDYCIAWFRQAPGKEREPVSCITTSDGSTYYADSVKGRFTISSDNAKNTVYLQMNRLKPEDTAVYYCAAYFGYGCYGGAQDYRAMDYWGKGTLVTVSS

SEQ ID NO: 73 - protein, 122 aa, Artificial Sequence
  antibody sequence
EVQLVESGGGLVQAGDSLRLSCAASGRTFSRYTMGWFRQAPGKEREFVAAISWSGGRTNFAGSVKGRFTISRDNAKNTVYLQMNSLKPEDTAVYYCAADWLPVPGRESYDYWGQGTQVTVSS

SEQ ID NO: 74 - protein, 130 aa, Artificial Sequence
  antibody sequence
EVQLVESGGGLVQAGGSLRLSCIASGRTFSNYAMGWFRQAPGKEREFVAAISWSGGMTDHADSVKGRFTISRDNAKNTVYLQMNSLKPEDTAVYYCAAAFAGDIPYGSSWYGDPTTYDYWGQGTQVTVSS

SEQ ID NO: 75 - protein, 124 aa, Artificial Sequence
  antibody sequence
EVQLVESGGGLVQAGGSLRLSCAASGRTSSTFSMAWFRQAPRKEREFVAAINWSGGSTRYADSVSDRFAISRDNAKNTVYLQMNNLKPEDTAVYYCAARRGGIYYSTQNDYDYWGQGTQVTVSS

SEQ ID NO: 76 - protein, 123 aa, Artificial Sequence
  antibody sequence
EVQLVESGGGLVQAGGSLRLSCAVSVRTFSDYRMGWFRQAPGKEREFVSTISWSGGLTYYADSVKGRFTISRDNSKNTLYLQMNSLKPEDTAVYYCAAGGGYAGGTYYHPEEWGQGTQVTVSS

SEQ ID NO: 77 - protein, 315 aa, Homo sapiens
MLSLLHASTLAVLGALCVYGAGHLEQPQISSTKTLSKTARLECVVSGITISATSVYWYRERPGEVIQFLVSISYDGTVRKESGIPSGKFEVDRIPETSTSTLTIHNVEKQDIATYYCALWEAQQELGKKIKVFGPGTKLIITDKQLDADVSPKPTIFLPSIAETKLQKAGTYLCLLEKFFPDVIKIHWEEKKSNTILGSQEGNTMKTNDTYMKFSWLTVPEKSLDKEHRCIVRHENNKNGVDQEIIFPPIKTDVITMDPKDNCSKDANDTLLLQLTNTSAYYMYLLLLLKSVVYFAIITCCLLRRTAFCCNGEKS

SEQ ID NO: 78 - protein, 292 aa, Homo sapiens [sequence omitted]

SEQ ID NO: 79 - protein, 4 aa, Artificial Sequence
  antibody sequence
NAMG

SEQ ID NO: 80 - protein, 16 aa, Artificial Sequence
  antibody sequence
VISSSGSTNYADSVKG

SEQ ID NO: 81 - protein, 10 aa, Artificial Sequence
  antibody sequence
HVAGFDEYNY

SEQ ID NO: 82 - protein, 118 aa, Artificial Sequence
  antibody sequence
QVQLVESGGGLVQAGGSLRLSCAASGSIFSINAMGWYRQAPGKQRDFLAVISSSGSTNYADSVKGRFTISRDNAKNTAYLQMNSLKVEDTAVYYCAAHVAGFDEYNYWGQGTQVTVSS

SEQ ID NO: 83 - protein, 5 aa, Artificial Sequence
  linker sequence
GGGGS

SEQ ID NO: 84 - protein, 254 aa, Artificial Sequence
  antibody sequence
QVQLVESGGGLVQAGGSLRLSCAASGSMFSDNVMGWYRQAPGKQRELVATIRTGGSTNYADSVKGRFTISRDNAKNTVYLQMNSLKPEDTAVYYCRHTIPVPSTPYDYWGQGTQVTVSSGGGGSEVQLVESGGGLVQAGGSLRLSCAASGRPFSNYAMGWFRQAPGKEREFVAAISWSGGSTSYADSVKGRFTISRDNAKNTVYLQMNSPKPEDTAIYYCAAQFSGADYGFGRLGIRGYEYDYWGQGTQVTVSS

SEQ ID NO: 85 - protein, 119 aa, Artificial Sequence
  antibody sequence
EVQLVESGGGLVQAGGSLRLSCAASGSMFSDNVMGWYRQAPGKQRELVATIRTGGSTNYADSVKGRFTISRDNAKNTVYLQMNSLKPEDTAVYYCRHTIPVPSTPYDYWGQGTQVTVSS

SEQ ID NO: 86 - protein, 130 aa, Artificial Sequence
  antibody sequence
EVQLLESGGGSVQPGGSLRLSCAASGRPFSNYAMSWFRQAPGKEREFVSAISWSGGSTSYADSVKGRFTISRDNSKNTLYLQMNSLRAEDTAVYYCAAQFSGADYGFGRLGIRGYEYDYWGQGTQVTVSS

SEQ ID NO: 87 - protein, 254 aa, Artificial Sequence
  antibody sequence
EVQLVESGGGLVQAGGSLRLSCAASGSMFSDNVMGWYRQAPGKQRELVATIRTGGSTNYADSVKGRFTISRDNAKNTVYLQMNSLKPEDTAVYYCRHTIPVPSTPYDYWGQGTQVTVSSGGGGSEVQLLESGGGSVQPGGSLRLSCAASGRPFSNYAMSWFRQAPGKEREFVSAISWSGGSTSYADSVKGRFTISRDNSKNTLYLQMNSLRAEDTAVYYCAAQFSGADYGFGRLGIRGYEYDYWGQGTQVTVSS

SEQ ID NO: 88 - protein, 130 aa, Artificial Sequence
  antibody sequence
EVQLLESGGGLVQPGGSLRLSCAASGRPFSNYAMSWFRQAPGKEREFVSAISWSGGSTSYADSVKGRFTISRDNSKNTLYLQMNSLRAEDTAVYYCAAQFSGADYGFGRLGIRGYEYDYWGQGTLVTVSS